European Patent Application EP 4 435 093 A2, published September 25, 2024. Title: UNIVERSAL DONOR CELLS. Applicant: CRISPR Therapeutics AG. The sequence listing filed with the application follows.

SEQUENCE LISTING (44 sequences)

SEQ ID NO: 1 - DNA, 20 bp, Homo sapiens
  source 1..20: mol_type = genomic DNA
gctactctctctttctggcc

SEQ ID NO: 2 - DNA, 20 bp, Homo sapiens
  source 1..20: mol_type = genomic DNA
ggccgagatgtctcgctccg

SEQ ID NO: 3 - DNA, 20 bp, Homo sapiens
  source 1..20: mol_type = genomic DNA
cgcgagcacagctaaggcca

SEQ ID NO: 4 - DNA, 20 bp, synthetic construct
  misc_feature 1..20: note = Synthesized
  source 1..20: mol_type = other DNA
cagacagcaaactcacccag

SEQ ID NO: 5 - DNA, 20 bp, synthetic construct
  misc_feature 1..20: note = Synthesized
  source 1..20: mol_type = other DNA
aaactttgtcccgaccctcc

SEQ ID NO: 6 - DNA, 638 bp, Homo sapiens
  source 1..638: mol_type = genomic DNA
cctagaatgagcgcccggtgtcccaagctggggcgcgcaccccagatcggcgggcgccgatgtacagacagcaaactcacccagtctagtgcatgccttcttaaacatcacgagactctagaaaaggaaactgaaaacgggaaagtccctctctctaacctggcactgcgtcgctggcttggagacaggtgacggtccctgcgggccttgtcctgattggctgggcacgcgtttaatataagtggaggcgtcgcgctggcgggcattcctgaagctgacagcattcgggccgagatgtctcgctccgtggccttagctgtgctcgcgctactctctctttctggcctggaggctatccagcgtgagtctctcctaccctcccgctctggtccttcctctcccgtctgcaccctctgtggccctcgctgtgctctctcgctccgtgacttcccttctccaagttctccttggtggcccgccgtggggctagtccagggctggatctcggggaagcggcggggtggcctgggagtggggaagggggtgcgcacccgggacgcgcgctacttgcccctttcggcggggagcaggggagacctttggcctacggcgacgggagggtcgggacaaagtttagg

SEQ ID NO: 7 - DNA, 20 bp, synthetic construct
  misc_feature 1..20: note = Synthesized
  source 1..20: mol_type = other DNA
tctgcagaaggctaccccta

SEQ ID NO: 8 - DNA, 24 bp, synthetic construct
  misc_feature 1..24: note = Synthesized
  source 1..24: mol_type = other DNA
tgctgtgtctaagacctctttcat

SEQ ID NO: 9 - DNA, 18 bp, synthetic construct
  misc_feature 1..18: note = Synthesized
  source 1..18: mol_type = other DNA
gatttggacctgcgagcg

SEQ ID NO: 10 - DNA, 22 bp, synthetic construct
  misc_feature 1..22: note = Synthesized
  source 1..22: mol_type = other DNA
caagcctggcaataaacaatga

SEQ ID NO: 11 - DNA, 15 bp, synthetic construct
  misc_feature 1..15: note = Synthesized
  source 1..15: mol_type = other DNA
ctgctgcctgaacat

SEQ ID NO: 12 - DNA, 130 bp, synthetic construct
  misc_feature 1..130: note = Synthesized
  source 1..130: mol_type = other DNA
cctgcaggcagctgcgcgctcgctcgctcactgaggccgcccgggcgtcgggcgacctttggtcgcccggcctcagtgagcgagcgagcgcgcagagagggagtggccaactccatcactaggggttcct

SEQ ID NO: 13 - DNA, 800 bp, Homo sapiens
  source 1..800: mol_type = genomic DNA
gttctagggtggaaactaagagaatgatgtacctagagggcgctggaagctctaaagccctagcagttactgcttttactattagtggtcgtttttttctcccccccgccccccgacaaatcaacagaacaaagaaaattacctaaacagcaaggacatagggaggaacttcttggcacagaactttccaaacactttttcctgaagggatacaagaagcaagaaaggtactctttcactaggaccttctctgagctgtcctcaggatgcttttgggactatttttcttacccagagaatggagaaaccctgcagggaattcccaagctgtagttataaacagaagttctccttctgctaggtagcattcaaagatcttaatcttctgggtttccgttttctcgaatgaaaaatgcaggtccgagcagttaactggctggggcaccattagcaagtcacttagcatctctggggccagtctgcaaagcgagggggcagccttaatgtgcctccagcctgaagtcctagaatgagcgcccggtgtcccaagctggggcgcgcaccccagatcggagggcgccgatgtacagacagcaaactcacccagtctagtgcatgccttcttaaacatcacgagactctaagaaaaggaaactgaaaacgggaaagtccctctctctaacctggcactgcgtcgctggcttggagacaggtgacggtccctgcgggccttgtcctgattggctgggcacgcgtttaatataagtggaggcgtcgcgctggcgggcattcctgaagct

SEQ ID NO: 14 - DNA, 380 bp, Cytomegalovirus
  source 1..380: mol_type = genomic DNA
gacattgattattgactagttattaatagtaatcaattacggggtcattagttcatagcccatatatggagttccgcgttacataacttacggtaaatggcccgcctggctgaccgcccaacgacccccgcccattgacgtcaataatgacgtatgttcccatagtaacgccaatagggactttccattgacgtcaatgggtggactatttacggtaaactgcccacttggcagtacatcaagtgtatcatatgccaagtacgccccctattgacgtcaatgacggtaaatggcccgcctggcattatgcccagtacatgaccttatgggactttcctacttggcagtacatctacgtattagtcatcgctattaccatg

SEQ ID NO: 15 - DNA, 276 bp, Gallus gallus
  source 1..276: mol_type = genomic DNA
tcgaggtgagccccacgttctgcttcactctccccatctcccccccctccccacccccaattttgtatttatttattttttaattattttgtgcagcgatgggggcggggggggggggggcgcgcgccaggcggggcggggcggggcgaggggcggggcggggcgaggcggagaggtgcggcggcagccaatcagagcggcgcgctccgaaagtttccttttatggcgaggcggcggcggcggcggccctataaaaagcgaagcgcgcggcgggcg

SEQ ID NO: 16 - DNA, 1009 bp, synthetic construct
  misc_feature 1..1009: note = Synthesized
  source 1..1009: mol_type = other DNA
ggagtcgctgcgttgccttcgccccgtgccccgctccgcgccgcctcgcgccgcccgccccggctctgactgaccgcgttactcccacaggtgagcgggcgggacggcccttctcctccgggctgtaattagcgcttggtttaatgacggctcgtttcttttctgtggctgcgtgaaagccttaaagggctccgggagggccctttgtgcgggggggagcggctcggggggtgcgtgcgtgtgtgtgtgcgtggggagcgccgcgtgcggcccgcgctgcccggcggctgtgagcgctgcgggcgcggcgcggggctttgtgcgctccgcgtgtgcgcgaggggagcgcggccgggggcggtgccccgcggtgcgggggggctgcgaggggaacaaaggctgcgtgcggggtgtgtgcgtgggggggtgagcagggggtgtgggcgcggcggtcgggctgtaacccccccctgcacccccctccccgagttgctgagcacggcccggcttcgggtgcggggctccgtgcggggcgtggcgcggggctcgccgtgccgggcggggggtggcggcaggtgggggtgccgggcggggcggggccgcctcgggccggggagggctcgggggaggggcgcggcggccccggagcgccggcggctgtcgaggcgcggcgagccgcagccattgccttttatggtaatcgtgcgagagggcgcagggacttcctttgtcccaaatctggcggagccgaaatctgggaggcgccgccgcaccccctctagcgggcgcgggcgaagcggtgcggcgccggcaggaaggaaatgggcggggagggccttcgtgcgtcgccgcgccgccgtccccttctccatctccagcctcggggctgccgcagggggacggctgccttcgggggggacggggcagggcggggttcggcttctggcgtgtgaccggcggctctagagcctctgctaaccatgttcatgccttcttctttttcctacag

SEQ ID NO: 17 - DNA, 873 bp, Homo sapiens
  source 1..873: mol_type = genomic DNA
atgaggatatttgctgtctttatattcatgacctactggcatttgctgaacgcatttactgtcacggttcccaaggacctatatgtggtagagtatggtagcaatatgacaattgaatgcaaattcccagtagaaaaacaattagacctggctgcactaattgtctattgggaaatggaggataagaacattattcaatttgtgcatggagaggaagacctgaaggttcagcatagtagctacagacagagggcccggctgttgaaggaccagctctccctgggaaatgctgcacttcagatcacagatgtgaaattgcaggatgcaggggtgtaccgctgcatgatcagctatggtggtgccgactacaagcgaattactgtgaaagtcaatgccccatacaacaaaatcaaccaaagaattttggttgtggatccagtcacctctgaacatgaactgacatgtcaggctgagggctaccccaaggccgaagtcatctggacaagcagtgaccatcaagtcctgagtggtaagaccaccaccaccaattccaagagagaggagaaacttttcaatgtgaccagcacactgagaatcaacacaacaactaatgagattttctactgcacttttaggagattagatcctgaggaaaaccatacagctgaattggtcatcccagaactacctctggcacatcctccaaatgaaaggactcacttggtaattctgggagccatcttattatgccttggtgtagcactgacattcatcttccgtttaagaaaagggagaatgatggatgtgaaaaaatgtggcatccaagatacaaactcaaagaagcaaagtgatacacatttggaggagacgtaa

SEQ ID NO: 18 - DNA, 225 bp, Bos taurus
  source 1..225: mol_type = genomic DNA
ctgtgccttctagttgccagccatctgttgtttgcccctcccccgtgccttccttgaccctggaaggtgccactcccactgtcctttcctaataaaatgaggaaattgcatcgcattgtctgagtaggtgtcattctattctggggggtggggtggggcaggacagcaagggggaggattgggaagacaatagcaggcatgctggggatgcggtgggctctatgg

SEQ ID NO: 19 - DNA, 800 bp, Homo sapiens
  source 1..800: mol_type = genomic DNA
ccagcgtgagtctctcctaccctcccgctctggtccttcctctcccgctctgcaccctctgtggccctcgctgtgctctctcgctccgtgacttcccttctccaagttctccttggtggcccgccgtggggctagtccagggctggatctcggggaagcggcggggtggcctgggagtggggaagggggtgcgcacccgggacgcgcgctacttgcccctttcggcggggagcaggggagacctttggcctacggcgacgggagggtcgggacaaagtttagggcgtcgataagcgtcagagcgccgaggttgggggagggtttctcttccgctctttcgcggggcctctggctcccccagcgcagctggagtgggggacgggtaggctcgtcccaaaggcgcggcgctgaggtttgtgaacgcgtggaggggcgcttggggtctgggggaggcgtcgcccgggtaagcctgtctgctgcggctctgcttcccttagactggagagctgtggacttcgtctaggcgcccgctaagttcgcatgtcctagcacctctgggtctatgtggggccacaccgtggggaggaaacagcacgcgacgtttgtagaatgcttggctgtgatacaaagcggtttcgaataattaacttatttgttcccatcacatgtcacttttaaaaaattataagaactacccgttattgacatctttctgtgtgccaaggactttatgtgctttgcgtcatttaattttgaaaacagttatcttccgccatagataactactatggttatcttct

SEQ ID NO: 20 - DNA, 141 bp, synthetic construct
  misc_feature 1..141: note = Synthesized
  source 1..141: mol_type = other DNA
aggaacccctagtgatggagttggccactccctctctgcgcgctcgctcgctcactgaggccgggcgaccaaaggtcgcccgacgcccgggctttgcccgggcggcctcagtgagcgagcgagcgcgcagctgcctgcagg

SEQ ID NO: 21 - DNA, 60 bp, Homo sapiens
  source 1..60: mol_type = genomic DNA
atgtctcgctccgtggccttagctgtgctcgcgctactctctctttctggcctggaggct

SEQ ID NO: 22 - DNA, 27 bp, Homo sapiens
  source 1..27: mol_type = genomic DNA
gtcatggcgccccgaaccctcttcctg

SEQ ID NO: 23 - DNA, 45 bp, synthetic construct
  misc_feature 1..45: note = Synthesized
  source 1..45: mol_type = other DNA
ggtggaggcggttcaggcggaggtggctctggcggtggcggatcg

SEQ ID NO: 24 - DNA, 297 bp, Homo sapiens
  source 1..297: mol_type = genomic DNA
atccagcgtactccaaagattcaggtttactcacgtcatccagcagagaatggaaagtcaaatttcctgaattgctatgtgtctgggtttcatccatccgacattgaagttgacttactgaagaatggagagagaattgaaaaagtggagcattcagacttgtctttcagcaaggactggtctttctatctcttgtactacactgaattcacccccactgaaaaagatgagtatgcctgccgtgtgaaccatgtgactttgtcacagcccaagatagttaagtgggatcgagacatg

SEQ ID NO: 25 - DNA, 60 bp, synthetic construct
  misc_feature 1..60: note = Synthesized
  source 1..60: mol_type = other DNA
ggtggtggtggttctggtggtggtggttctggcggcggcggctccggtggtggtggatcc

SEQ ID NO: 26 - DNA, 1011 bp, Homo sapiens
  source 1..1011: mol_type = genomic DNA
ggctcccactccttgaagtatttccacacttccgtgtcccggcccggccgcggggagccccgcttcatctctgtgggctacgtggacgacacccagttcgtgcgcttcgacaacgacgccgcgagtccgaggatggtgccgcgggcgccgtggatggagcaggaggggtcagagtattgggaccgggagacacggagcgccagggacaccgcacagattttccgagtgaatctgcggacgctgcgcggctactacaatcagagcgaggccgggtctcacaccctgcagtggatgcatggctgcgagctggggcccgacgggcgcttcctccgcgggtatgaacagttcgcctacgacggcaaggattatctcaccctgaatgaggacctgcgctcctggaccgcggtggacacggcggctcagatctccgagcaaaagtcaaatgatgcctctgaggcggagcaccagagagcctacctggaagacacatgcgtggagtggctccacaaatacctggagaaggggaaggagacgctgcttcacctggagcccccaaagacacacgtgactcaccaccccatctctgaccatgaggccaccctgaggtgctgggccctgggcttctaccctgcggagatcacactgacctggcagcaggatggggagggccatacccaggacacggagctcgtggagaccaggcctgcaggggatggaaccttccagaagtgggcagctgtggtggtgccttctggagaggagcagagatacacgtgccatgtgcagcatgaggggctacccgagcccgtcaccctgagatggaagccggcttcccagcccaccatccccatcgtgggcatcattgctggcctggttctccttggatctgtggtctctggagctgtggttgctgctgtgatatggaggaagaagagctcaggtggaaaaggagggagctactctaaggctgagtggagcgacagtgcccaggggtctgagtctcacagcttg

SEQ ID NO: 27 - DNA, 67 bp, synthetic construct
  misc_feature 1..67: note = Synthesized
  misc_feature 3..32: note = n is a, c, g, or t
  misc_feature 43..58: note = n is a, c, g, or t
  misc_feature 63: note = n is a, c, g, or t
  source 1..67: mol_type = other DNA
ctnnnnnnnnnnnnnnnnnnnnnnnnnnnnnncgctccgtggnnnnnnnnnnnnnnnngctanacgt

SEQ ID NO: 28 - DNA, 64 bp, synthetic construct
  misc_feature 1..64: note = Synthesized
  misc_feature 3..32: note = n is a, c, g, or t
  misc_feature 45..60: note = n is a, c, g, or t
  source 1..64: mol_type = other DNA
ctnnnnnnnnnnnnnnnnnnnnnnnnnnnnnncgcgctacttagnnnnnnnnnnnnnnnngcta

SEQ ID NO: 29 - DNA, 63 bp, synthetic construct
  misc_feature 1..63: note = Synthesized
  misc_feature 3..32: note = n is a, c, g, or t
  misc_feature 44..59: note = n is a, c, g, or t
  source 1..63: mol_type = other DNA
ctnnnnnnnnnnnnnnnnnnnnnnnnnnnnnncgcttccgtggnnnnnnnnnnnnnnnngcta

SEQ ID NO: 30 - DNA, 26 bp, synthetic construct
  misc_feature 1..26: note = Synthesized
  misc_feature 7..22: note = n is a, c, g, or t
  source 1..26: mol_type = other DNA
ctaaggnnnnnnnnnnnnnnnngcta

SEQ ID NO: 31 - skipped

SEQ ID NO: 32 - DNA, 61 bp, synthetic construct
  misc_feature 1..61: note = Synthesized
  misc_feature 3..32: note = n is a, c, g, or t
  misc_feature 42..57: note = n is a, c, g, or t
  source 1..61: mol_type = other DNA
ctnnnnnnnnnnnnnnnnnnnnnnnnnnnnnncgcccgtggnnnnnnnnnnnnnnnngcta

SEQ ID NO: 33 - DNA, 7133 bp, synthetic construct
  misc_feature 1..7133: note = Synthesized
  source 1..7133: mol_type = other DNA
cctgcaggcagctgcgcgctcgctcgctcactgaggccgcccgggcgtcgggcgacctttggtcgcccggcctcagtgagcgagcgagcgcgcagagagggagtggccaactccatcactaggggttcctgcggccgcacgcgtgttctagggtggaaactaagagaatgatgtacctagagggcgctggaagctctaaagccctagcagttactgcttttactattagtggtcgtttttttctcccccccgccccccgacaaatcaacagaacaaagaaaattacctaaacagcaaggacatagggaggaacttcttggcacagaactttccaaacactttttcctgaagggatacaagaagcaagaaaggtactctttcactaggaccttctctgagctgtcctcaggatgcttttgggactatttttcttacccagagaatggagaaaccctgcagggaattcccaagctgtagttataaacagaagttctccttctgctaggtagcattcaaagatcttaatcttctgggtttccgttttctcgaatgaaaaatgcaggtccgagcagttaactggctggggcaccattagcaagtcacttagcatctctggggccagtctgcaaagcgagggggcagccttaatgtgcctccagcctgaagtcctagaatgagcgcccggtgtcccaagctggggcgcgcaccccagatcggagggcgccgatgtacagacagcaaactcacccagtctagtgcatgccttcttaaacatcacgagactctaagaaaaggaaactgaaaacgggaaagtccctctctctaacctggcactgcgtcgctggcttggagacaggtgacggtccctgcgggccttgtcctgattggctgggcacgcgtttaatataagtggaggcgtcgcgctggcgggcattcctgaagctaagcttgtggacgatatcgaattcgcacgacattgattattgactagttattaatagtaatcaattacggggtcattagttcatagcccatatatggagttccgcgttacataacttacggtaaatggcccgcctggctgaccgcccaacgacccccgcccattgacgtcaataatgacgtatgttcccatagtaacgccaatagggactttccattgacgtcaatgggtggactatttacggtaaactgcccacttggcagtacatcaagtgtatcatatgccaagtacgccccctattgacgtcaatgacggtaaatggcccgcctggcattatgcccagtacatgaccttatgggactttcctacttggcagtacatctacgtattagtcatcgctattaccatgggtcgaggtgagccccacgttctgcttcactctccccatctcccccccctccccacccccaattttgtatttatttattttttaattattttgtgcagcgatgggggcggggggggggggggcgcgcgccaggcggggcggggcggggcgaggggcggggcggggcgaggcggagaggtgcggcggcagccaatcagagcggcgcgctccgaaagtttccttttatggcgaggcggcggcggcggcggccctataaaaagcgaagcgcgcggcgggcgggagtcgctgcgttgccttcgccccgtgccccgctccgcgccgcctcgcgccgcccgccccggctctgactgaccgcgttactcccacaggtgagcgggcgggacggcccttctcctccgggctgtaattagcgcttggtttaatgacggctcgtttcttttctgtggctgcgtgaaagccttaaagggctccgggagggccctttgtgcgggggggagcggctcggggggtgcgtgcgtgtgtgtgtgcgtggggagcgccgcgtgcggcccgcgctgcccggcggctgtgagcgctgcgggcgcggcgcggggctttgtgcgctccgcgtgtgcgcgaggggagcgcggccgggggcggtgccccgcggtgcgggggggctgcgaggggaacaaaggctgcgtgcggggtgtgtgcgtgggggggtgagcagggggtgtgggcgcggcggtcgggctgtaacccccccctgcacccccctccccgagttgctgagcacggcccggcttcgggtgcggggctccgtgcggggcgtggcgcggggctcgccgtgccgggcggggggtggcggcaggtgggggtgccgggcggggcggggccgcctcgggccggggagggctcgggggaggggcgcggcggccccggagcgccggcggctgtcgaggcgcggcgagccgcagccattgccttttatggtaatcgtgcgagagggcgcagggacttcctttgtcccaaatctggcggagccgaaatctgggaggcgccgccgcaccccctctagcgggcgcgggcgaagcggtgcggcgccggcaggaaggaaatgggcggggagggccttcgtgcgtcgccgcgccgccgtccccttctccatctccagcctcggggctgccgcagggggacggctgccttcgggggggacggggcagggcggggttcggcttctggcgtgtgaccggcggctctagagcctctgctaaccatgttcatgccttcttctttttcctacaggggggatccgtttatctgcagaattcgcccttgacgtcgccaccatgaggatatttgctgtctttatattcatgacctactggcatttgctgaacgcatttactgtcacggttcccaaggacctatatgtggtagagtatggtagcaatatgacaattgaatgcaaattcccagtagaaaaacaattagacctggctgcactaattgtctattgggaaatggaggataagaacattattcaatttgtgcatggagaggaagacctgaaggttcagcatagtagctacagacagagggcccggctgttgaaggaccagctctccctgggaaatgctgcacttcagatcacagatgtgaaattgcaggatgcaggggtgtaccgctgcatgatcagctatggtggtgccgactacaagcgaattactgtgaaagtcaatgccccatacaacaaaatcaaccaaagaattttggttgtggatccagtcacctctgaacatgaactgacatgtcaggctgagggctaccccaaggccgaagtcatctggacaagcagtgaccatcaagtcctgagtggtaagaccaccaccaccaattccaagagagaggagaaacttttcaatgtgaccagcacactgagaatcaacacaacaactaatgagattttctactgcacttttaggagattagatcctgaggaaaaccatacagctgaattggtcatcccagaactacctctggcacatcctccaaatgaaaggactcacttggtaattctgggagccatcttattatgccttggtgtagcactgacattcatcttccgtttaagaaaagggagaatgatggatgtgaaaaaatgtggcatccaagatacaaactcaaagaagcaaagtgatacacatttggaggagacgtaaccgctgatcagcctcgactgtgccttctagttgccagccatctgttgtttgcccctcccccgtgccttccttgaccctggaaggtgccactcccactgtcctttcctaataaaatgaggaaattgcatcgcattgtctgagtaggtgtcattctattctggggggtggggtggggcaggacagcaagggggaggattgggaagacaatagcaggcatgctggggatgcggtgggctctatgggtcgacccagcgtgagtctctcctaccctcccgctctggtccttcctctcccgctctgcaccctctgtggccctcgctgtgctctctcgctccgtgacttcccttctccaagttctccttggtggcccgccgtggggctagtccagggctggatctcggggaagcggcggggtggcctgggagtggggaagggggtgcgcacccgggacgcgcgctacttgcccctttcggcggggagcaggggagacctttggcctacggcgacgggagggtcgggacaaagtttagggcgtcgataagcgtcagagcgccgaggttgggggagggtttctcttccgctctttcgcggggcctctggctcccccagcgcagctggagtgggggacgggtaggctcgtcccaaaggcgcggcgctgaggtttgtgaacgcgtggaggggcgcttggggtctgggggaggcgtcgcccgggtaagcctgtctgctgcggctctgcttcccttagactggagagctgtggacttcgtctaggcgcccgctaagttcgcatgtcctagcacctctgggtctatgtggggccacaccgtggggaggaaacagcacgcgacgtttgtagaatgcttggctgtgatacaaagcggtttcgaataattaacttatttgttcccatcacatgtcacttttaaaaaattataagaactacccgttattgacatctttctgtgtgccaaggactttatgtgctttgcgtcatttaattttgaaaacagttatcttccgccatagataactactatggttatcttctggtaaccacgtgcggaccgaggctgcagcgtcgtcctccctaggaacccctagtgatggagttggccactccctctctgcgcgctcgctcgctcactgaggccgggcgaccaaaggtcgcccgacgcccgggctttgcccgggcggcctcagtgagcgagcgagcgcgcagctgcctgcaggggcgcctgatgcggtattttctccttacgcatctgtgcggtatttcacaccgcatacgtcaaagcaaccatagtacgcgccctgtagcggcgcattaagcgcggcgggtgtggtggttacgcgcagcgtgaccgctacacttgccagcgccctagcgcccgctcctttcgctttcttcccttcctttctcgccacgttcgccggctttccccgtcaagctctaaatcgggggctccctttagggttccgatttagtgctttacggcacctcgaccccaaaaaacttgatttgggtgatggttcacgtagtgggccatcgccctgatagacggtttttcgccctttgacgttggagtccacgttctttaatagtggactcttgttccaaactggaacaacactcaaccctatctcgggctattcttttgatttataagggattttgccgatttcggcctattggttaaaaaatgagctgatttaacaaaaatttaacgcgaattttaacaaaatattaacgtttacaattttatggtgcactctcagtacaatctgctctgatgccgcatagttaagccagccccgacacccgccaacacccgctgacgcgccctgacgggcttgtctgctcccggcatccgcttacagacaagctgtgaccgtctccgggagctgcatgtgtcagaggttttcaccgtcatcaccgaaacgcgcgagacgaaagggcctcgtgatacgcctatttttataggttaatgtcatgaacaataaaactgtctgcttacataaacagtaatacaaggggtgttatgagccatattcaacgggaaacgtcgaggccgcgattaaattccaacatggatgctgatttatatgggtataaatgggctcgcgataatgtcgggcaatcaggtgcgacaatctatcgcttgtatgggaagcccgatgcgccagagttgtttctgaaacatggcaaaggtagcgttgccaatgatgttacagatgagatggtcagactaaactggctgacggaatttatgcctcttccgaccatcaagcattttatccgtactcctgatgatgcatggttactcaccactgcgatccccggaaaaacagcattccaggtattagaagaatatcctgattcaggtgaaaatattgttgatgcgctggcagtgttcctgcgccggttgcattcgattcctgtttgtaattgtccttttaacagcgatcgcgtatttcgtctcgctcaggcgcaatcacgaatgaataacggtttggttgatgcgagtgattttgatgacgagcgtaatggctggcctgttgaacaagtctggaaagaaatgcataaacttttgccattctcaccggattcagtcgtcactcatggtgatttctcacttgataaccttatttttgacgaggggaaattaataggttgtattgatgttggacgagtcggaatcgcagaccgataccaggatcttgccatcctatggaactgcctcggtgagttttctccttcattacagaaacggctttttcaaaaatatggtattgataatcctgatatgaataaattgcagtttcatttgatgctcgatgagtttttctaatctcatgaccaaaatcccttaacgtgagttttcgttccactgagcgtcagaccccgtagaaaagatcaaaggatcttcttgagatcctttttttctgcgcgtaatctgctgcttgcaaacaaaaaaaccaccgctaccagcggtggtttgtttgccggatcaagagctaccaactctttttccgaaggtaactggcttcagcagagcgcagataccaaatactgtccttctagtgtagccgtagttaggccaccacttcaagaactctgtagcaccgcctacatacctcgctctgctaatcctgttaccagtggctgctgccagtggcgataagtcgtgtcttaccgggttggactcaagacgatagttaccggataaggcgcagcggtcgggctgaacggggggttcgtgcacacagcccagcttggagcgaacgacctacaccgaactgagatacctacagcgtgagctatgagaaagcgccacgcttcccgaagggagaaaggcggacaggtatccggtaagcggcagggtcggaacaggagagcgcacgagggagcttccagggggaaacgcctggtatctttatagtcctgtcgggtttcgccacctctgacttgagcgtcgatttttgtgatgctcgtcaggggggcggagcctatggaaaaacgccagcaacgcggcctttttacggttcctggccttttgctggccttttgctcacatgt

SEQ ID NO: 34 - DNA, 7763 bp, synthetic construct
  misc_feature 1..7763: note = Synthesized
  source 1..7763: mol_type = other DNA
cctgcaggcagctgcgcgctcgctcgctcactgaggccgcccgggcgtcgggcgacctttggtcgcccggcctcagtgagcgagcgagcgcgcagagagggagtggccaactccatcactaggggttcctgcggccgcacgcgtgttctagggtggaaactaagagaatgatgtacctagagggcgctggaagctctaaagccctagcagttactgcttttactattagtggtcgtttttttctcccccccgccccccgacaaatcaacagaacaaagaaaattacctaaacagcaaggacatagggaggaacttcttggcacagaactttccaaacactttttcctgaagggatacaagaagcaagaaaggtactctttcactaggaccttctctgagctgtcctcaggatgcttttgggactatttttcttacccagagaatggagaaaccctgcagggaattcccaagctgtagttataaacagaagttctccttctgctaggtagcattcaaagatcttaatcttctgggtttccgttttctcgaatgaaaaatgcaggtccgagcagttaactggctggggcaccattagcaagtcacttagcatctctggggccagtctgcaaagcgagggggcagccttaatgtgcctccagcctgaagtcctagaatgagcgcccggtgtcccaagctggggcgcgcaccccagatcggagggcgccgatgtacagacagcaaactcacccagtctagtgcatgccttcttaaacatcacgagactctaagaaaaggaaactgaaaacgggaaagtccctctctctaacctggcactgcgtcgctggcttggagacaggtgacggtccctgcgggccttgtcctgattggctgggcacgcgtttaatataagtggaggcgtcgcgctggcgggcattcctgaagctaagcttgtggacgatatcgaattcgcacgacattgattattgactagttattaatagtaatcaattacggggtcattagttcatagcccatatatggagttccgcgttacataacttacggtaaatggcccgcctggctgaccgcccaacgacccccgcccattgacgtcaataatgacgtatgttcccatagtaacgccaatagggactttccattgacgtcaatgggtggactatttacggtaaactgcccacttggcagtacatcaagtgtatcatatgccaagtacgccccctattgacgtcaatgacggtaaatggcccgcctggcattatgcccagtacatgaccttatgggactttcctacttggcagtacatctacgtattagtcatcgctattaccatgggtcgaggtgagccccacgttctgcttcactctccccatctcccccccctccccacccccaattttgtatttatttattttttaattattttgtgcagcgatgggggcggggggggggggggcgcgcgccaggcggggcggggcggggcgaggggcggggcggggcgaggcggagaggtgcggcggcagccaatcagagcggcgcgctccgaaagtttccttttatggcgaggcggcggcggcggcggccctataaaaagcgaagcgcgcggcgggcgggagtcgctgcgttgccttcgccccgtgccccgctccgcgccgcctcgcgccgcccgccccggctctgactgaccgcgttactcccacaggtgagcgggcgggacggcccttctcctccgggctgtaattagcgcttggtttaatgacggctcgtttcttttctgtggctgcgtgaaagccttaaagggctccgggagggccctttgtgcgggggggagcggctcggggggtgcgtgcgtgtgtgtgtgcgtggggagcgccgcgtgcggcccgcgctgcccggcggctgtgagcgctgcgggcgcggcgcggggctttgtgcgctccgcgtgtgcgcgaggggagcgcggccgggggcggtgccccgcggtgcgggggggctgcgaggggaacaaaggctgcgtgcggggtgtgtgcgtgggggggtgagcagggggtgtgggcgcggcggtcgggctgtaacccccccctgcacccccctccccgagttgctgagcacggcccggcttcgggtgcggggctccgtgcggggcgtggcgcggggctcgccgtgccgggcggggggtggcggcaggtgggggtgccgggcggggcggggccgcctcgggccggggagggctcgggggaggggcgcggcggccccggagcgccggcggctgtcgaggcgcggcgagccgcagccattgccttttatggtaatcgtgcgagagggcgcagggacttcctttgtcccaaatctggcggagccgaaatctgggaggcgccgccgcaccccctctagcgggcgcgggcgaagcggtgcggcgccggcaggaaggaaatgggcggggagggccttcgtgcgtcgccgcgccgccgtccccttctccatctccagcctcggggctgccgcagggggacggctgccttcgggggggacggggcagggcggggttcggcttctggcgtgtgaccggcggctctagagcctctgctaaccatgttcatgccttcttctttttcctacaggggggatccgtttatctgcagaattcgcccttgacgtcgccaccatgtctcgctccgtggccttagctgtgctcgcgctactctctctttctggcctggaggctgtcatggcgccccgaaccctcttcctgggtggaggcggttcaggcggaggtggctctggcggtggcggatcgatccagcgtactccaaagattcaggtttactcacgtcatccagcagagaatggaaagtcaaatttcctgaattgctatgtgtctgggtttcatccatccgacattgaagttgacttactgaagaatggagagagaattgaaaaagtggagcattcagacttgtctttcagcaaggactggtctttctatctcttgtactacactgaattcacccccactgaaaaagatgagtatgcctgccgtgtgaaccatgtgactttgtcacagcccaagatagttaagtgggatcgagacatgggtggtggtggttctggtggtggtggttctggcggcggcggctccggtggtggtggatccggctcccactccttgaagtatttccacacttccgtgtcccggcccggccgcggggagccccgcttcatctctgtgggctacgtggacgacacccagttcgtgcgcttcgacaacgacgccgcgagtccgaggatggtgccgcgggcgccgtggatggagcaggaggggtcagagtattgggaccgggagacacggagcgccagggacaccgcacagattttccgagtgaatctgcggacgctgcgcggctactacaatcagagcgaggccgggtctcacaccctgcagtggatgcatggctgcgagctggggcccgacgggcgcttcctccgcgggtatgaacagttcgcctacgacggcaaggattatctcaccctgaatgaggacctgcgctcctggaccgcggtggacacggcggctcagatctccgagcaaaagtcaaatgatgcctctgaggcggagcaccagagagcctacctggaagacacatgcgtggagtggctccacaaatacctggagaaggggaaggagacgctgcttcacctggagcccccaaagacacacgtgactcaccaccccatctctgaccatgaggccaccctgaggtgctgggccctgggcttctaccctgcggagatcacactgacctggcagcaggatggggagggccatacccaggacacggagctcgtggagaccaggcctgcaggggatggaaccttccagaagtgggcagctgtggtggtgccttctggagaggagcagagatacacgtgccatgtgcagcatgaggggctacccgagcccgtcaccctgagatggaagccggcttcccagcccaccatccccatcgtgggcatcattgctggcctggttctccttggatctgtggtctctggagctgtggttgctgctgtgatatggaggaagaagagctcaggtggaaaaggagggagctactctaaggctgagtggagcgacagtgcccaggggtctgagtctcacagcttgtaaccgctgatcagcctcgactgtgccttctagttgccagccatctgttgtttgcccctcccccgtgccttccttgaccctggaaggtgccactcccactgtcctttcctaataaaatgaggaaattgcatcgcattgtctgagtaggtgtcattctattctggggggtggggtggggcaggacagcaagggggaggattgggaagacaatagcaggcatgctggggatgcggtgggctctatgggtcgacccagcgtgagtctctcctaccctcccgctctggtccttcctctcccgctctgcaccctctgtggccctcgctgtgctctctcgctccgtgacttcccttctccaagttctccttggtggcccgccgtggggctagtccagggctggatctcggggaagcggcggggtggcctgggagtggggaagggggtgcgcacccgggacgcgcgctacttgcccctttcggcggggagcaggggagacctttggcctacggcgacgggagggtcgggacaaagtttagggcgtcgataagcgtcagagcgccgaggttgggggagggtttctcttccgctctttcgcggggcctctggctcccccagcgcagctggagtgggggacgggtaggctcgtcccaaaggcgcggcgctgaggtttgtgaacgcgtggaggggcgcttggggtctgggggaggcgtcgcccgggtaagcctgtctgctgcggctctgcttcccttagactggagagctgtggacttcgtctaggcgcccgctaagttcgcatgtcctagcacctctgggtctatgtggggccacaccgtggggaggaaacagcacgcgacgtttgtagaatgcttggctgtgatacaaagcggtttcgaataattaacttatttgttcccatcacatgtcacttttaaaaaattataagaactacccgttattgacatctttctgtgtgccaaggactttatgtgctttgcgtcatttaattttgaaaacagttatcttccgccatagataactactatggttatcttctggtaaccacgtgcggaccgaggctgcagcgtcgtcctccctaggaacccctagtgatggagttggccactccctctctgcgcgctcgctcgctcactgaggccgggcgaccaaaggtcgcccgacgcccgggctttgcccgggcggcctcagtgagcgagcgagcgcgcagctgcctgcaggggcgcctgatgcggtattttctccttacgcatctgtgcggtatttcacaccgcatacgtcaaagcaaccatagtacgcgccctgtagcggcgcattaagcgcggcgggtgtggtggttacgcgcagcgtgaccgctacacttgccagcgccctagcgcccgctcctttcgctttcttcccttcctttctcgccacgttcgccggctttccccgtcaagctctaaatcgggggctccctttagggttccgatttagtgctttacggcacctcgaccccaaaaaacttgatttgggtgatggttcacgtagtgggccatcgccctgatagacggtttttcgccctttgacgttggagtccacgttctttaatagtggactcttgttccaaactggaacaacactcaaccctatctcgggctattcttttgatttataagggattttgccgatttcggcctattggttaaaaaatgagctgatttaacaaaaatttaacgcgaattttaacaaaatattaacgtttacaattttatggtgcactctcagtacaatctgctctgatgccgcatagttaagccagccccgacacccgccaacacccgctgacgcgccctgacgggcttgtctgctcccggcatccgcttacagacaagctgtgaccgtctccgggagctgcatgtgtcagaggttttcaccgtcatcaccgaaacgcgcgagacgaaagggcctcgtgatacgcctatttttataggttaatgtcatgaacaataaaactgtctgcttacataaacagtaatacaaggggtgttatgagccatattcaacgggaaacgtcgaggccgcgattaaattccaacatggatgctgatttatatgggtataaatgggctcgcgataatgtcgggcaatcaggtgcgacaatctatcgcttgtatgggaagcccgatgcgccagagttgtttctgaaacatggcaaaggtagcgttgccaatgatgttacagatgagatggtcagactaaactggctgacggaatttatgcctcttccgaccatcaagcattttatccgtactcctgatgatgcatggttactcaccactgcgatccccggaaaaacagcattccaggtattagaagaatatcctgattcaggtgaaaatattgttgatgcgctggcagtgttcctgcgccggttgcattcgattcctgtttgtaattgtccttttaacagcgatcgcgtatttcgtctcgctcaggcgcaatcacgaatgaataacggtttggttgatgcgagtgattttgatgacgagcgtaatggctggcctgttgaacaagtctggaaagaaatgcataaacttttgccattctcaccggattcagtcgtcactcatggtgatttctcacttgataaccttatttttgacgaggggaaattaataggttgtattgatgttggacgagtcggaatcgcagaccgataccaggatcttgccatcctatggaactgcctcggtgagttttctccttcattacagaaacggctttttcaaaaatatggtattgataatcctgatatgaataaattgcagtttcatttgatgctcgatgagtttttctaatctcatgaccaaaatcccttaacgtgagttttcgttccactgagcgtcagaccccgtagaaaagatcaaaggatcttcttgagatcctttttttctgcgcgtaatctgctgcttgcaaacaaaaaaaccaccgctaccagcggtggtttgtttgccggatcaagagctaccaactctttttccgaaggtaactggcttcagcagagcgcagataccaaatactgtccttctagtgtagccgtagttaggccaccacttcaagaactctgtagcaccgcctacatacctcgctctgctaatcctgttaccagtggctgctgccagtggcgataagtcgtgtcttaccgggttggactcaagacgatagttaccggataaggcgcagcggtcgggctgaacggggggttcgtgcacacagcccagcttggagcgaacgacctacaccgaactgagatacctacagcgtgagctatgagaaagcgccacgcttcccgaagggagaaaggcggacaggtatccggtaagcggcagggtcggaacaggagagcgcacgagggagcttccagggggaaacgcctggtatctttatagtcctgtcgggtttcgccacctctgacttgagcgtcgatttttgtgatgctcgtcaggggggcggagcctatggaaaaacgccagcaacgcggcctttttacggttcctggccttttgctggccttttgctcacatgt

SEQ ID NO: 35 - DNA, 20 bp, Homo sapiens
  source 1..20: mol_type = genomic DNA
tataagtggaggcgtcgcgc

SEQ ID NO: 36 - DNA, 20 bp, Homo sapiens
  source 1..20: mol_type = genomic DNA
gagtagcgcgagcacagcta

SEQ ID NO: 37 - DNA, 20 bp, Homo sapiens
  source 1..20: mol_type = genomic DNA
actggacgcgtcgcgctggc

SEQ ID NO: 38 - DNA, 20 bp, Homo sapiens
  source 1..20: mol_type = genomic DNA
aagtggaggcgtcgcgctgg

SEQ ID NO: 39 - DNA, 20 bp, Homo sapiens
  source 1..20: mol_type = genomic DNA
ggccacggagcgagacatct

SEQ ID NO: 40 - DNA, 20 bp, Homo sapiens
  source 1..20: mol_type = genomic DNA
gcccgaatgctgtcagcttc

SEQ ID NO: 41 - DNA, 20 bp, Homo sapiens
  source 1..20: mol_type = genomic DNA
ctcgcgctactctctctttc

SEQ ID NO: 42 - DNA, 20 bp, Homo sapiens
  source 1..20: mol_type = genomic DNA
tcctgaagctgacagcattc

SEQ ID NO: 43 - DNA, 20 bp, Homo sapiens
  source 1..20: mol_type = genomic DNA
ttcctgaagctgacagcatt

SEQ ID NO: 44 - DNA, 20 bp, Homo sapiens
  source 1..20: mol_type = genomic DNA
actctctctttctggcctgg